European Patent Application EP 4 450 513 A1, published October 23, 2024. Title: RECOMBINANT PARTICLE PROTEIN PRODUCT SUITABLE FOR INDUSTRIAL PRODUCTION AND PREPARATION METHOD THEREFOR. Applicant: Yantai Patronus Biotech Co., Ltd. The sequence listing filed with the application follows.

SEQUENCE LISTING (1 sequence)

SEQ ID NO: 1 - protein, 309 aa, synthetic construct
DSATHIKFSKRDEDGKELAGATMELRDSSGKTISTWISDGQVKDFYLYPGKYTFVETAAPDGYEVATAITFTVNEQGQVTVNGKATKGDAHIGGSGGSGGSGGSMKMEELFKKHKIVAVLRANSVEEAKKKALAVFLGGVHLIEITFTVPDADTVIKELSFLKEMGAIIGAGTVTSVEQARKAVESGAEFIVSPHLDEEISQFAKEKGVFYMPGVMTPTELVKAMKLGHTILKLFPGEVVGPQFVKAMKGPFPNVKFVPTGGVNLDNVCEWFKAGVLAVGVGSALVKGTPVEVAEKAKAFVEKIRGCTE